European Patent Specification EP 2 971 023 B1, published December 11, 2024. Title: Methods of using natural and engineered organisms to produce small molecules for industrial application. Applicant: Kiverdi, inc. The sequence listing filed with the application follows.

SEQUENCE LISTING (22 sequences)

SEQ ID NO: 1 - protein, 416 aa, Cupriavidus necator
MALIVHKYGGTSMGSTERIKNVAKRVAKWHRAGHRVVVVPSAMSGETNRLLGLAKEISPQPNPRELDMLASTGEQASVALLAIALHGEDIDAVSYTGWQVPVKTDSAYTKARIESIDDERILADLDAGRVVVITGFQGIDDDGNITTLGRGGSDTSAVAIAAAIEADECLIYTDVDGVYTTDPRVVEDARRLDQITFEEMLEMASLGSKVLQIRSVEFAGKYRVKTRVLSSLTDPLMPLEQEMHSGTLITFEEDSTMEAAVISGIAFARDEAKITVLGVPDKPGIAYQILGPVADANIDVDMIIQNQSVDGKTDFTFTVPRGEYQRALAILNDGVKSHIGAGSVSGDPKVSKVSVVGVGMRSHVGIASKMFRTLSEEGINIQMISTSEIKISVLIDEKYMELAVRALHKAFELEQA

SEQ ID NO: 2 - protein, 304 aa, Cupriavidus necator
MNNKLTAADLRGIFPAIPTPVTADDRIDQDATRKLMAYLLANGVSGVVPLGGTGEYGALAREERVRMAALCVEAAAGQVPVIPGVLDPGFHDALDAGKAFAGVGASALMVLTPYYTSPTQQGIRDYFLRYADASPVPVMIYEIPYRTRIAIAPEVLHELSRHENIIGMKACNTDMYHFLKVVAGVDDSFSVFSGEDSLFPLHMAGGARGGVVVTASVLPRTWRAIYELGVAGNTAQAVRLHRELIPLLDLAFSETNPGPLKSVLDLVGVTAPKVLAPLVAPAPGLQAQLRAELTQRLQAEAALA

SEQ ID NO: 3 - protein, 216 aa, Ralstonia eutropha
MNSLPDTASLALSIALQGLALSLGLIVAIGAQNAFVLRQGLRRQHVGSVVLFCAAADALLIAAGVMGMAQALGDRPGLARALAVAGSVFLAIYGWQALQRARQSHQLKAADGVDGLGRGAVLAQAAAFTLLNPHVYLDTVLLVGSIGAQQPAALRGWFVAGASAASLFWFGLLGFGARWLAPWFARPKAWRVLDGVIAMTMFVLSALLVRHVFNAV

SEQ ID NO: 4 - protein, 293 aa, Ralstonia eutropha
MSILINKDTKVITQGITGKTGQFHTRGCRDYANGKNCFVAGVNPKKAGEDFEGIPIYASVKDAKAQTGATVSVIYVPPAGAAAAIWEAVDADLDLVVCITEGIPVRDMMEVKDRMRRENKKTLLLGPNCPGLITPDEIKIGIMPGHIHRKGRIGVVSRSGTLTYEAVGQLTALGLGQSSAVGIGGDPINGLKHIDVMKMFNDDPETDAVVMIGEIGGPDEANAAYWIKDNMKKPVVGFIAGVTAPPGKRMGHAGALISGGADTAQAKLEIMEACGITVTKNPSEMARLLKAKL

SEQ ID NO: 5 - protein, 389 aa, Ralstonia eutropha
MNIHEYQGKEILRKYNVPVPRGIPAFSVAEALKAAEELGGPVWVVKAQIHAGGRGKGGGVKVAKSIDDVKTYATNILGMQLVTHQTGPEGKKVNRLLIEEGADIKKELYVSLVVDRVSQKIALMASSEGGMDIEEVAAHTPEKIHTLIIEPSTGLTDADADDIARKIGVPDASVAQARQALQGLYKAFYDTDASLAEINPLILTGEGKVIALDAKFNFDSNALFRHPEIVAYRDLDEEDANEIEASKFDLAYISLDGNIGCLVNGAGLAMATMDTIKLFGGEPANFLDVGGGATTEKVTEAFKLMLKNPNVEAILVNIFGGIMRCDVIAEGVISASKAVNLTVPLVVRMKGTNEDLGKKMLADSGLPIIAADTMEEAAQKVVAAAAGKK

SEQ ID NO: 6 - protein, 370 aa, Ralstonia eutropha
MSGNTLGLLFTVTTFGESHGPAIGAVVDGCPPGMDLTEADIQGDLDRRKPGTSRHVTQRKEPDQVEILSGVFEGKTTGTPICLLIRNTDQRSKDYGNIVETFRPGHADYTYWQKYGIRDYRGGGRSSARLTAPVVAAGAVAKKWLREQFGTEIRGYMSKLGEIEVPFSDWSHVPENPFFAANADIVPELETYMDALRRDGDSVGARIEVVASNVPVGLGEPLFDRLDADIAHAMMGLNAVKGVEIGAGFKSVEQRGSEHGDELTAQGFRGNNAGGILGGISTGQDITVSLAIKPTSSIRTPRESIDKAGNAATVETFGRHDPCVGIRATPIAEALLALVLVDHALRHRAQCGDVKVDTPRIPAQAPGQPG

SEQ ID NO: 7 - protein, 304 aa, Ralstonia eutropha
MKPITLFGAPTDVGASTRGCTMGPEALRIADIVPALARMGLDVSDAGNIAGPVNPLAPPVQGLRHLDEVVAWNRGVFEASTRILQAGRMPVLLGGDHCLAVGSVSAVARHCREAGRKLVVLWLDAHADANIGTSTPTGNMHGMPVACLCGDGPTPLTTLGGQPPAVRPEEIRQVGIRSVDAQEKLRLHALGLKVFDMRYIDEYGMRQTMEQALAGVDDDTHLHVSFDVDFIDSAIAPGVGTTVLGGPTYRETQLCMEMIADTGRLSSLDVMELNPACDVRNETARLVVDFLESLFGKSTLLRAR

SEQ ID NO: 8 - protein, 756 aa, Ralstonia eutropha
MKFRFPVIIIDEDFRSENISGSGIRALAEAIEKEGMEVMGLTSYGDLTSFAQQSSRASTFIVSIDDDEFVTADDQPEAAAIEKLRAFVNEVRRRNTDLPIFLYGETRTSRHIPNDILRELHGFIHMFEDTPEFVARHIIREAKVYLDTLAPPFFKALIDYAQDSSYSWHCPGHSGGVAFLKSPVGQVFHQFFGENMLRADVCNAVDELGQLLDHTGPVAASERNAARIFNSDHMFFVTNGTSTSNKMVWHANVAPGDIVVVDRNCHKSILHAIMMTGAIPVFLMPTRNHYGIIGPIPKSEFDPETIRRKIANHPFASKAKNQKPRILTITQGTYDGVLYNAEQIKEMLASEIDTLHFDEAWLPHAAFHEFYHNMHAIGRDRPRSKDALVFATQSTHKLLAGLSQASQILVQDSETRKLDRYRFNEAYLMHTSTSPQYAIIASCDVAAAMMEAPGGPALVEESIQEALDFRRAMRKVEGDFEAGNNGDWWFKVWGPDTLNDEGMPEREQWMLKANERWHGFGDLADGFNLLDPIKATIITPGLDVDGEFSDRGIPAAIVTKYLAEHGIIIEKTGLYSFFIMFTIGITKGRWNSLVTELQQFKDDYDQNQPLWRVLPEFVGKHPQYERMGLRDLCDAVHSVYKANDVARVTTEMYLSDMEPAMKPSDAWSMMAHREIERVPVDDLEGRVTAILLTPYPPGIPLLIPGERFNRTIVQYLKFAREFNKLFPGFETDVHGLVEEEVDGRKAYFVDCVKQGS

SEQ ID NO: 9 - protein, 454 aa, Rhodobacter capsulatus
MKTIIEPFRIKSVEPIRLTSRPERERLARAAGYNLFGLHSDDVLIDLLTDSGTGAMSSLQWAAVMQGDESYAGSPSFFRFEAAVQNLMPFKHIIPTHQGRAAEAILFSIFGGKGRRIPSNTHFDTTRGNIEASGATGDDLVIAEGKDPQNLHPFKGNMDLARLEAYLEAHHAEVPLVMITITNNAGGGQPVSLANIRAVADLAHRYGKPFVIDGCRFAENAWFIKTREEGQADRSIPEIVRDCFAVADGMTMSAKKDAFGNIGGWLALNDDDLAEEARGHLIRTEGFPTYGGLAGRDLDALAQGLVEIVDEDYLRYRIRTHQYIVERLDAMGVPVVKPAGGHAVFIDARAWLSHIPPLEYPGQALAVALYEIAGVRSCEIGTAMFGRQPDGSEKPAAMDLVRLAFPRRTYTQSHADYIVEAFEELAATKDALRGYRIVKEPKLMRHFTCRFEKL

SEQ ID NO: 10 - protein, 645 aa, Sulfurospirillum multivorans
MNNQKSTIDTSKFDNVLDSSKTFVDHEPDSSKEIQRNTPQKTMPFSDQIGNYQRNRGIPAYSYDESKVYIVGSGIAGLSAAFYLIRDGRIPAQNITFLEKLSVEGGSMDGAGDAREGYIIRGGREMDMTYENLWDLFQDVPAVELPEPYSVLDEYRLLNDNDSNYSKARFIHNKGHITDFSKFGLSKKDQLAIIKLLLKKKEDLDDVTIQDYFSESFLASDFWTLWRTMFAFENWHSVLECKLYMHRFLHVLDGMKDLSALVFPKYNQYDTFIAPLRKLLQEKGVQFQFDTLVEDLEITMTHNEKIVENIVTIHNETSSKIAVGRDDYVIVTTGSMTEDTFYGDNHNAPIISIDNTTSGQSSGWKLWKNLAKKSEVFGKPEKFCSTIEHSSWESATLTCKPSAFVEKLKKLSVNDPYSGKTVTGGIITITDSNWLMSFTCNRQPHFIEQPDDILVIWLYALFMDKEGNYVKKPMPECSGDEILTELCYHLGIKDDLENVLKNTIVRTAFMPYITSMFMPRAKGDRPRIVPKGCKNLGLIGQFVETNNDIVFTMESSIRTARIAVYTLLNLNKQVPDINPLQYDIRQLLKAVKSLNDDQPFIGEGILRKFLKDTYYEYILPPMSKESEQESSFMEHIEKIKEWILR

SEQ ID NO: 11 - DNA, 20 bp, artificial sequence
  synthetic polynucleotide
atggctctcatcgttcacaa

SEQ ID NO: 12 - DNA, 19 bp, artificial sequence
  synthetic polynucleotide
tcacgcctgttccagttcg

SEQ ID NO: 13 - DNA, 25 bp, artificial sequence
  synthetic polynucleotide
gttctgggacgaggtgacgctgcag

SEQ ID NO: 14 - DNA, 24 bp, artificial sequence
  synthetic polynucleotide
gtatgcggccaggttgcgtgccag

SEQ ID NO: 15 - DNA, 28 bp, artificial sequence
  synthetic polynucleotide
atgaactccctgcctgacaccgcttccc

SEQ ID NO: 16 - DNA, 30 bp, artificial sequence
  synthetic polynucleotide
tcacactgcgttgaatacgtgacgcaccag

SEQ ID NO: 17 - DNA, 28 bp, artificial sequence
  synthetic polynucleotide
tgaagcgcccaggaagcattctggacag

SEQ ID NO: 18 - DNA, 25 bp, artificial sequence
  synthetic polynucleotide
cgcgcgaagaacccgcccgtttcac

SEQ ID NO: 19 - DNA, 26 bp, artificial sequence
  synthetic polynucleotide
cctcgtcgcctacgtcgaacgcatgc

SEQ ID NO: 20 - DNA, 25 bp, artificial sequence
  synthetic polynucleotide
cagcacgccgatctgcacggcgttg

SEQ ID NO: 21 - DNA, 27 bp, artificial sequence
  synthetic polynucleotide
ccgagtgggaaggctatgtgacgctgg

SEQ ID NO: 22 - DNA, 24 bp, artificial sequence
  synthetic polynucleotide
gtggtagtggcagccgagccggtg